European Patent Application EP 4 183 803 A1, published May 24, 2023. Title: FUSION PROTEIN COMPRISING EXTRACELLULAR DOMAIN OF IgE Fc RECEPTOR ALPHA SUBUNIT AND ANTI-IL-4 RECEPTOR ANTIBODY AND USE THEREOF. Applicant: GI Innovation, Inc. The sequence listing filed with the application follows.

SEQUENCE LISTING (32 sequences)

SEQ ID NO: 1 - protein, 19 aa, Artificial Sequence
  mIgG signal
MEWSWVFLFFLSVTTGVHS

SEQ ID NO: 2 - protein, 180 aa, Artificial Sequence
  FceRIa ECD
VPQKPKVSLNPPWNRIFKGENVTLTCNGNNFFEVSSTKWFHNGSLSEETNSSLNIVNAKFEDSGEYKCQHQQVNESEPVYLEVFSDWLLLQASAEVVMEGQPLFLRCHGWRNWDVYKVIYYKDGEALKYWYENHNISITNATVEDSGTYYCTGKVWQLDYESEPLNITVIKAPREKYWLQ

SEQ ID NO: 3 - protein, 30 aa, Artificial Sequence
  NL028 hinge linker
GSGGGGSGGGGSGGGGSAESKYGPPCPPCP

SEQ ID NO: 4 - protein, 216 aa, Artificial Sequence
  hIgG4Fc
APEAAGGPSVFLFPPKPKDQLMISRTPEVTCVVVDVSQEDPEVQFNWYVDGVEVHNAKTKPREEQFNSTYRVVSVLTVLHQDWLNGKEYKCKVSNKGLPSSIEKTISKAKGQPREPQVYTLPPSQEEMTKNQVSLTCLVKGFYPSDIAVEWESNGQPENNYKTTPPVLDSDGSFFLYSRLTVDKSRWQEGNVFSCSVLHEALHNHYTQKSLSLSLG

SEQ ID NO: 5 - protein, 12 aa, Artificial Sequence
  (G4S)2GG linker
GGGGSGGGGSGG

SEQ ID NO: 6 - protein, 257 aa, Artificial Sequence
  Anti-IL-4R scFv
EVQLVESGGGLEQPGGSLRLSCAGSGFTFRDYAMTWVRQAPGKCLEWVSSISGSGGNTYYADSVKGRFTISRDNSKNTLYLQMNSLRAEDTAVYYCAKDRLSITIRPRYYGLDVWGQGTTVTVSSGGGGSGGGGSGGGGSGGGGSDIVMTQSPLSLPVTPGEPASISCRSSQSLLYSIGYNYLDWYLQKSGQSPQLLIYLGSNRASGVPDRFSGSGSGTDFTLKISRVEAEDVGFYYCMQALQTPYTFGCGTKLEIK

SEQ ID NO: 7 - protein, 125 aa, Artificial Sequence
  Anti-IL-4R_heavy chain
EVQLVESGGGLEQPGGSLRLSCAGSGFTFRDYAMTWVRQAPGKCLEWVSSISGSGGNTYYADSVKGRFTISRDNSKNTLYLQMNSLRAEDTAVYYCAKDRLSITIRPRYYGLDVWGQGTTVTVSS

SEQ ID NO: 8 - protein, 112 aa, Artificial Sequence
  Anti-IL-4R_light chain
DIVMTQSPLSLPVTPGEPASISCRSSQSLLYSIGYNYLDWYLQKSGQSPQLLIYLGSNRASGVPDRFSGSGSGTDFTLKISRVEAEDVGFYYCMQALQTPYTFGCGTKLEIK

SEQ ID NO: 9 - protein, 20 aa, Artificial Sequence
  HC-LC linker
GGGGSGGGGSGGGGSGGGGS

SEQ ID NO: 10 - protein, 695 aa, Artificial Sequence
  GI-305(FceRIa ECD-Fc-anti-IL-4R scFv)
VPQKPKVSLNPPWNRIFKGENVTLTCNGNNFFEVSSTKWFHNGSLSEETNSSLNIVNAKFEDSGEYKCQHQQVNESEPVYLEVFSDWLLLQASAEVVMEGQPLFLRCHGWRNWDVYKVIYYKDGEALKYWYENHNISITNATVEDSGTYYCTGKVWQLDYESEPLNITVIKAPREKYWLQGSGGGGSGGGGSGGGGSAESKYGPPCPPCPAPEAAGGPSVFLFPPKPKDQLMISRTPEVTCVVVDVSQEDPEVQFNWYVDGVEVHNAKTKPREEQFNSTYRVVSVLTVLHQDWLNGKEYKCKVSNKGLPSSIEKTISKAKGQPREPQVYTLPPSQEEMTKNQVSLTCLVKGFYPSDIAVEWESNGQPENNYKTTPPVLDSDGSFFLYSRLTVDKSRWQEGNVFSCSVLHEALHNHYTQKSLSLSLGGGGGSGGGGSGGEVQLVESGGGLEQPGGSLRLSCAGSGFTFRDYAMTWVRQAPGKCLEWVSSISGSGGNTYYADSVKGRFTISRDNSKNTLYLQMNSLRAEDTAVYYCAKDRLSITIRPRYYGLDVWGQGTTVTVSSGGGGSGGGGSGGGGSGGGGSDIVMTQSPLSLPVTPGEPASISCRSSQSLLYSIGYNYLDWYLQKSGQSPQLLIYLGSNRASGVPDRFSGSGSGTDFTLKISRVEAEDVGFYYCMQALQTPYTFGCGTKLEIK

SEQ ID NO: 11 - DNA, 540 bp, Artificial Sequence
  Polynucleotides coding FceRIa ECD
gtgcctcagaaacccaaagtgtctctgaaccctccttggaaccggatcttcaagggcgagaacgtgaccctgacctgcaacggcaacaacttcttcgaggtgtcctccaccaagtggttccacaacggctccctgtccgaggaaacaaactccagcctgaacatcgtgaacgccaagttcgaggactccggcgagtacaagtgccagcaccagcaagtgaacgagtccgagcctgtgtacctggaagtgttctccgactggctgctgctccaggcttctgccgaggttgtgatggaaggccagcctctgttcctgagatgtcacggctggcggaactgggacgtgtacaaagtgatctactacaaggacggcgaggccctgaagtattggtacgagaaccacaacatctccatcaccaacgccaccgtggaagattccggcacctactactgcaccggcaaagtgtggcagctggactacgagagcgagcctctgaacatcaccgtgatcaaggcccctagagagaagtactggctgcaa

SEQ ID NO: 12 - DNA, 90 bp, Artificial Sequence
  Polynucleotides coding NL028 hinge linker
ggatctggcggcggaggttctggcggaggtggaagcggtggcggaggatctgctgagtctaagtatggccctccttgtcctccatgtcct

SEQ ID NO: 13 - DNA, 648 bp, Artificial Sequence
  Polynucleotides coding hIgG4Fc
gctccagaagctgctggcgggccctccgtgtttctgttccctccaaagcctaaggaccagctgatgatctctcggacacccgaagtgacctgcgtggtggtggatgtgtctcaagaggaccctgaggtgcagttcaattggtacgtggacggcgtggaagtgcacaacgccaagaccaagcctagagaggaacagttcaactccacctacagagtggtgtccgtgctgaccgtgctgcaccaggattggctgaacggcaaagagtacaagtgcaaggtgtccaacaagggcctgccttccagcatcgaaaagaccatctccaaggccaagggccagcctagggaaccccaggtttacaccctgcctccaagccaagaggaaatgaccaagaaccaggtgtccctgacctgcctggtcaagggcttctacccttccgacattgccgtggaatgggagagcaatggccagcctgagaacaactacaagaccacacctcctgtgctggactccgacggctccttctttctgtactcccgcctgaccgtggacaagtccagatggcaagagggcaacgtgttctcctgctctgtgctgcacgaggccctgcacaatcactacacccagaagtccctcagcctgtcccttggc

SEQ ID NO: 14 - DNA, 36 bp, Artificial Sequence
  Polynucleotides coding (G4S)2GG linker
ggaggcggtggatcaggtggcggaggatctggcgga

SEQ ID NO: 15 - DNA, 771 bp, Artificial Sequence
  Polynucleotides coding Anti-IL-4R scFv
gaagtgcagctggttgaatctggcggcggattggaacagcctggcggatctctgagactgtcttgtgccggctctggcttcaccttcagagactacgctatgacctgggtccgacaggctcctggcaaatgtctggaatgggtgtcctccatctctggctctggcggcaatacctactacgccgactctgtgaagggcagattcaccatcagccgggacaactccaagaacaccctgtacctccagatgaactccctgagagccgaggacaccgccgtgtactactgcgccaaggacagactgtccatcaccatccggcctcggtactacggactggatgtttggggccagggcaccacagtgacagtgtcctccggaggcggaggaagtggcggcggaggatcaggcggtggtggatctggcggaggcggttctgacattgtgatgacccagtctccactgagcctgcctgtgacacctggcgagcctgcttccatctcttgccggtcatctcagtccctgctgtactccatcggctacaactacctggactggtatctccagaagtccggacagtctccccagctgctgatctacctgggctccaatagagcctccggcgtgcccgatagattctccggatctggctctggcaccgacttcaccctgaagatctccagagtggaagccgaggacgtgggcttctactactgtatgcaggccctccagacaccttacacctttggctgtggcaccaagctggaaatcaag

SEQ ID NO: 16 - DNA, 375 bp, Artificial Sequence
  Polynucleotides coding Anti-IL-4R_heavy chain
gaagtgcagctggttgaatctggcggcggattggaacagcctggcggatctctgagactgtcttgtgccggctctggcttcaccttcagagactacgctatgacctgggtccgacaggctcctggcaaatgtctggaatgggtgtcctccatctctggctctggcggcaatacctactacgccgactctgtgaagggcagattcaccatcagccgggacaactccaagaacaccctgtacctccagatgaactccctgagagccgaggacaccgccgtgtactactgcgccaaggacagactgtccatcaccatccggcctcggtactacggactggatgtttggggccagggcaccacagtgacagtgtcctcc

SEQ ID NO: 17 - DNA, 336 bp, Artificial Sequence
  Polynucleotides coding Anti-IL-4R_light chain
gacattgtgatgacccagtctccactgagcctgcctgtgacacctggcgagcctgcttccatctcttgccggtcatctcagtccctgctgtactccatcggctacaactacctggactggtatctccagaagtccggacagtctccccagctgctgatctacctgggctccaatagagcctccggcgtgcccgatagattctccggatctggctctggcaccgacttcaccctgaagatctccagagtggaagccgaggacgtgggcttctactactgtatgcaggccctccagacaccttacacctttggctgtggcaccaagctggaaatcaag

SEQ ID NO: 18 - DNA, 57 bp, Artificial Sequence
  Polynucleotides coding mIgG signal
atggaatggtcctgggtgttcctgttcttcctgtccgtgaccaccggcgtgcactct

SEQ ID NO: 19 - DNA, 2085 bp, Artificial Sequence
  Polynucleotides coding GI-305
gtgcctcagaaacccaaagtgtctctgaaccctccttggaaccggatcttcaagggcgagaacgtgaccctgacctgcaacggcaacaacttcttcgaggtgtcctccaccaagtggttccacaacggctccctgtccgaggaaacaaactccagcctgaacatcgtgaacgccaagttcgaggactccggcgagtacaagtgccagcaccagcaagtgaacgagtccgagcctgtgtacctggaagtgttctccgactggctgctgctccaggcttctgccgaggttgtgatggaaggccagcctctgttcctgagatgtcacggctggcggaactgggacgtgtacaaagtgatctactacaaggacggcgaggccctgaagtattggtacgagaaccacaacatctccatcaccaacgccaccgtggaagattccggcacctactactgcaccggcaaagtgtggcagctggactacgagagcgagcctctgaacatcaccgtgatcaaggcccctagagagaagtactggctgcaaggatctggcggcggaggttctggcggaggtggaagcggtggcggaggatctgctgagtctaagtatggccctccttgtcctccatgtcctgctccagaagctgctggcgggccctccgtgtttctgttccctccaaagcctaaggaccagctgatgatctctcggacacccgaagtgacctgcgtggtggtggatgtgtctcaagaggaccctgaggtgcagttcaattggtacgtggacggcgtggaagtgcacaacgccaagaccaagcctagagaggaacagttcaactccacctacagagtggtgtccgtgctgaccgtgctgcaccaggattggctgaacggcaaagagtacaagtgcaaggtgtccaacaagggcctgccttccagcatcgaaaagaccatctccaaggccaagggccagcctagggaaccccaggtttacaccctgcctccaagccaagaggaaatgaccaagaaccaggtgtccctgacctgcctggtcaagggcttctacccttccgacattgccgtggaatgggagagcaatggccagcctgagaacaactacaagaccacacctcctgtgctggactccgacggctccttctttctgtactcccgcctgaccgtggacaagtccagatggcaagagggcaacgtgttctcctgctctgtgctgcacgaggccctgcacaatcactacacccagaagtccctcagcctgtcccttggcggaggcggtggatcaggtggcggaggatctggcggagaagtgcagctggttgaatctggcggcggattggaacagcctggcggatctctgagactgtcttgtgccggctctggcttcaccttcagagactacgctatgacctgggtccgacaggctcctggcaaatgtctggaatgggtgtcctccatctctggctctggcggcaatacctactacgccgactctgtgaagggcagattcaccatcagccgggacaactccaagaacaccctgtacctccagatgaactccctgagagccgaggacaccgccgtgtactactgcgccaaggacagactgtccatcaccatccggcctcggtactacggactggatgtttggggccagggcaccacagtgacagtgtcctccggaggcggaggaagtggcggcggaggatcaggcggtggtggatctggcggaggcggttctgacattgtgatgacccagtctccactgagcctgcctgtgacacctggcgagcctgcttccatctcttgccggtcatctcagtccctgctgtactccatcggctacaactacctggactggtatctccagaagtccggacagtctccccagctgctgatctacctgggctccaatagagcctccggcgtgcccgatagattctccggatctggctctggcaccgacttcaccctgaagatctccagagtggaagccgaggacgtgggcttctactactgtatgcaggccctccagacaccttacacctttggctgtggcaccaagctggaaatcaag

SEQ ID NO: 20 - protein, 8 aa, Artificial Sequence
  HCDR1
GFTFRDYA

SEQ ID NO: 21 - protein, 8 aa, Artificial Sequence
  HCDR2
ISGSGGNT

SEQ ID NO: 22 - protein, 18 aa, Artificial Sequence
  HCDR3
AKDRLSITIRPRYYGLDV

SEQ ID NO: 23 - protein, 11 aa, Artificial Sequence
  LCDR1
QSLLYSIGYNY

SEQ ID NO: 24 - protein, 3 aa, Artificial Sequence
  LCDR2
LGS

SEQ ID NO: 25 - protein, 9 aa, Artificial Sequence
  LCDR3
MQALQTPYT

SEQ ID NO: 26 - protein, 125 aa, Artificial Sequence [sequence omitted]

SEQ ID NO: 27 - protein, 112 aa, Artificial Sequence [sequence omitted]

SEQ ID NO: 28 - protein, 30 aa, Artificial Sequence
  GI-301 hinge linker
RNTGRGGEEKKGSKEKEEQEERETKTPECP

SEQ ID NO: 29 - protein, 215 aa, Artificial Sequence
  GI-301 modified Fc
SHTQPLGVFLFPPKPKDTLMISRTPEVTCVVVDVSQEDPEVQFNWYVDGVEVHNAKTKPREEQFNSTYRVVSVLTVLHQDWLNGKEYKCKVSNKGLPSSIEKTISKAKGQPREPQVYTLPPSQEEMTKNQVSLTCLVKGFYPSDIAVEWESNGQPENNYKTTPPVLDSDGSFFLYSRLTVDKSRWQEGNVFSCSVMHEALHNHYTQKSLSLSLGK

SEQ ID NO: 30 - DNA, 1275 bp, Artificial Sequence
  Polynucleotides coding GI-301
gtgccccagaagcccaaggtgagcctgaaccctccctggaacagaatcttcaagggcgagaacgtgaccctgacctgcaacggcaacaacttcttcgaggtgagcagcaccaagtggttccacaatggcagcctgagcgaggagaccaacagctccctgaacatcgtgaacgccaagttcgaggacagcggcgagtacaagtgccagcaccagcaggtgaacgagagcgagcccgtgtacctggaggtgttcagcgactggctgctgctgcaggccagcgccgaggtggtgatggagggccagcccctgttcctgagatgccacggctggagaaactgggacgtgtacaaggtgatctactacaaggatggcgaggccctgaagtactggtacgagaaccacaacatctccatcaccaacgccaccgtggaggacagcggcacctactactgcacaggcaaggtgtggcagctggactacgagagcgagcccctgaacatcaccgtgatcaaggctcccagagagaagtactggctgcagaggaacaccggcagaggaggcgaggaaaagaaaggaagcaaggagaaggaggagcaggaggaaagagaaaccaagacccccgagtgccccagccacacccagcccctgggcgtgttcctgttcccccccaagcccaaggacaccctgatgatcagcagaacccccgaggtgacctgcgtggtcgtggatgtgagccaggaagatcccgaagtgcagttcaactggtacgtggatggcgtggaagtgcacaacgccaagaccaagcccagagaagagcagttcaactccacctacagagtggtgagcgtgctgaccgtgctgcaccaggactggctgaacggcaaggagtacaagtgcaaggtgtccaacaaaggcctgcccagctccatcgagaagaccatcagcaaagccaaaggccagcccagagaaccccaggtgtacaccctgcctcccagccaggaagagatgaccaagaaccaggtgtccctgacctgcctggtgaaaggcttctaccccagcgacatcgccgtggagtgggaaagcaacggccagcccgagaacaattacaagacaacccctcccgtgctggatagcgatggcagcttctttctgtacagcagactgaccgtggacaagagcagatggcaggaaggcaacgtgttcagctgcagcgtgatgcacgaagccctgcacaaccactacacccagaagagcctgtccctgagcctgggcaag

SEQ ID NO: 31 - DNA, 1278 bp, Artificial Sequence
  Polynucleotides coding GI-305CN
gtgcctcagaaacccaaagtgtctctgaaccctccttggaaccggatcttcaagggcgagaacgtgaccctgacctgcaacggcaacaacttcttcgaggtgtcctccaccaagtggttccacaacggctccctgtccgaggaaacaaactccagcctgaacatcgtgaacgccaagttcgaggactccggcgagtacaagtgccagcaccagcaagtgaacgagtccgagcctgtgtacctggaagtgttctccgactggctgctgctccaggcttctgccgaggttgtgatggaaggccagcctctgttcctgagatgtcacggctggcggaactgggacgtgtacaaagtgatctactacaaggacggcgaggccctgaagtattggtacgagaaccacaacatctccatcaccaacgccaccgtggaagattccggcacctactactgcaccggcaaagtgtggcagctggactacgagagcgagcctctgaacatcaccgtgatcaaggcccctagagagaagtactggctgcaaggatctggcggcggaggttctggcggaggtggaagcggtggcggaggatctgctgagtctaagtatggccctccttgtcctccatgtcctgctccagaagctgctggcgggccctccgtgtttctgttccctccaaagcctaaggaccagctgatgatctctcggacacccgaagtgacctgcgtggtggtggatgtgtctcaagaggaccctgaggtgcagttcaattggtacgtggacggcgtggaagtgcacaacgccaagaccaagcctagagaggaacagttcaactccacctacagagtggtgtccgtgctgaccgtgctgcaccaggattggctgaacggcaaagagtacaagtgcaaggtgtccaacaagggcctgccttccagcatcgaaaagaccatctccaaggccaagggccagcctagggaaccccaggtttacaccctgcctccaagccaagaggaaatgaccaagaaccaggtgtccctgacctgcctggtcaagggcttctacccttccgacattgccgtggaatgggagagcaatggccagcctgagaacaactacaagaccacacctcctgtgctggactccgacggctccttctttctgtactcccgcctgaccgtggacaagtccagatggcaagagggcaacgtgttctcctgctctgtgctgcacgaggccctgcacaatcactacacccagaagtccctcagcctgtcccttggc

SEQ ID NO: 32 - DNA, 1494 bp, Artificial Sequence
  Polynucleotides coding GI-305C1
gctgagtctaagtatggccctccttgtcctccatgtcctgctccagaagctgctggcgggccctccgtgtttctgttccctccaaagcctaaggaccagctgatgatctctcggacacccgaagtgacctgcgtggtggtggatgtgtctcaagaggaccctgaggtgcagttcaattggtacgtggacggcgtggaagtgcacaacgccaagaccaagcctagagaggaacagttcaactccacctacagagtggtgtccgtgctgaccgtgctgcaccaggattggctgaacggcaaagagtacaagtgcaaggtgtccaacaagggcctgccttccagcatcgaaaagaccatctccaaggccaagggccagcctagggaaccccaggtttacaccctgcctccaagccaagaggaaatgaccaagaaccaggtgtccctgacctgcctggtcaagggcttctacccttccgacattgccgtggaatgggagagcaatggccagcctgagaacaactacaagaccacacctcctgtgctggactccgacggctccttctttctgtactcccgcctgaccgtggacaagtccagatggcaagagggcaacgtgttctcctgctctgtgctgcacgaggccctgcacaatcactacacccagaagtccctcagcctgtcccttggcggaggcggtggatcaggtggcggaggatctggcggagaagtgcagctggttgaatctggcggcggattggaacagcctggcggatctctgagactgtcttgtgccggctctggcttcaccttcagagactacgctatgacctgggtccgacaggctcctggcaaatgtctggaatgggtgtcctccatctctggctctggcggcaatacctactacgccgactctgtgaagggcagattcaccatcagccgggacaactccaagaacaccctgtacctccagatgaactccctgagagccgaggacaccgccgtgtactactgcgccaaggacagactgtccatcaccatccggcctcggtactacggactggatgtttggggccagggcaccacagtgacagtgtcctccggaggcggaggaagtggcggcggaggatcaggcggtggtggatctggcggaggcggttctgacattgtgatgacccagtctccactgagcctgcctgtgacacctggcgagcctgcttccatctcttgccggtcatctcagtccctgctgtactccatcggctacaactacctggactggtatctccagaagtccggacagtctccccagctgctgatctacctgggctccaatagagcctccggcgtgcccgatagattctccggatctggctctggcaccgacttcaccctgaagatctccagagtggaagccgaggacgtgggcttctactactgtatgcaggccctccagacaccttacacctttggctgtggcaccaagctggaaatcaag